European Patent Specification EP 3 402 821 B1, published August 23, 2023. Title: Novel PSMA binding antibody and uses thereof. Applicant: Deutsches Krebsforschungszentrum Stiftung des oeffentlichen Rechts Eberhard Karls Universitaet Tuebingen. The sequence listing filed with the application follows.

SEQUENCE LISTING (16 sequences)

SEQ ID NO: 1 - protein, 119 aa, Artificial Sequence
  murine 10B3 antibody heavy chain variable region
QVQLQESGGGLVKPGGSLKLSCAASGFTFSDFYMYWVRQTPEKRLEWVATISDGGGYTSYPDSVKGRFTISRDIAKNNLYLQMNSLKSEDTAKYYCARGLWLRDALDYWGQGTSVTVSS

SEQ ID NO: 2 - protein, 109 aa, Artificial Sequence
  murine 10B3 antibody light chain variable region
EIVLTQSPITMAAFLGERITITCSASSSISSNYLHWYQQKPGFSPKLLIYRTSNLASGVPIRFSGSGSGTSYSLTIGTMEAEDVATYYCQQGSYIPFTFGSGTKLEIKR

SEQ ID NO: 3 - protein, 10 aa, Artificial Sequence
  CDR-H1 of 10B3 antibody
GFTFSDFYMY

SEQ ID NO: 4 - protein, 17 aa, Artificial Sequence
  CDR-H2 of 10B3 antibody
TISDGGGYTSYPDSVKG

SEQ ID NO: 5 - protein, 10 aa, Artificial Sequence
  CDR-H3 of 10B3 antibody
GLWLRDALDY

SEQ ID NO: 6 - protein, 12 aa, Artificial Sequence
  CDR-L1 of 10B3 antibody
SASSSISSNYLH

SEQ ID NO: 7 - protein, 7 aa, Artificial Sequence
  CDR-L2 of 10B3 antibody
RTSNLAS

SEQ ID NO: 8 - protein, 9 aa, Artificial Sequence
  CDR-L3 of 10B3 antibody
QQGSYIPFT

SEQ ID NO: 9 - protein, 119 aa, Artificial Sequence
  humanized 10B3 antibody heavy chain variable region
QVQLVESGGGLVKPGGSLRLSCAASGFTFSDFYMYWIRQAPGKGLEWVATISDGGGYTSYPDSVKGRFTISRDNAKNSLYLQMNSLRAEDTAVYYCARGLWLRDALDYWGQGTTVTVSS

SEQ ID NO: 10 - protein, 109 aa, Artificial Sequence
  humanized 10B3 antibody light chain variable region
EIVLTQSPATLSLSPGERATLSCSASSSISSNYLHWYQQKPGQAPRLLIYRTSNLASGIPARFSGSGSGTDYTLTISRLEPEDFAVYYCQQGSYIPFTFGQGTKLEIKR

SEQ ID NO: 11 - protein, 714 aa, Artificial Sequence
  heavy chain of h10B3xhUCHT1 bispecific IgGsc format antibody
METDTLLLWVLLLWVPGSTGQVQLVESGGGLVKPGGSLRLSCAASGFTFSDFYMYWIRQAPGKGLEWVATISDGGGYTSYPDSVKGRFTISRDNAKNSLYLQMNSLRAEDTAVYYCARGLWLRDALDYWGQGTTVTVSSASTKGPSVFPLAPSSKSTSGGTAALGCLVKDYFPEPVTVSWNSGALTSGVHTFPAVLQSSGLYSLSSVVTVPSSSLGTQTYICNVNHKPSNTKVDKKVEPKSCDKTHTCPPCPAPPVAGPSVFLFPPKPKDTLMISRTPEVTCVVVGVSHEDPEVKFNWYVDGVEVHNAKTKPREEQYNSTYRVVSVLTVLHQDWLNGKEYKCKVSNKQLPSPIEKTISKAKGQPREPQVYTLPPSRDELTKNQVSLTCLVKGFYPSDIAVEWESNGQPENNYKTTPPVLDSDGSFFLYSKLTVDKSRWQQGNVFSCSVMHEALHNHYTQKSLSLSPGKSGDIQMTQSPSSLSASVGDRVTITCRASQDIRNYLNWYQQKPGKAPKLLIYYTSRLESGVPSRFSGSGSGTDYTLTISSLQPEDFATYYCQQGNTLPWTFGQGTKVEIKGGGGSGGGGSGGGGSEVQLVESGGGLVQPGGSLRLSCAASGYSFTGYTMNWVRQAPGKGLEWVALINPYKGVSTYNQKFKDRFTISVDKSKNTAYLQMNSLRAEDTAVYYCARSGYYGDSDWYFDVWGQGTLVTVSS

SEQ ID NO: 12 - protein, 606 aa, Artificial Sequence
  heavy chain of h10B3xOKT3 bispecific Fabsc format antibody
METDTLLLWVLLLWVPGSTGQVQLVESGGGLVKPGGSLRLSCAASGFTFSDFYMYWIRQAPGKGLEWVATISDGGGYTSYPDSVKGRFTISRDNAKNSLYLQMNSLRAEDTAVYYCARGLWLRDALDYWGQGTTVTVSSASTKGPSVFPLAPSSKSTSGGTAALGCLVKDYFPEPVTVSWNSGALTSGVHTFPAVLQSSGLYSLSSVVTVPSSSLGTQTYICNVNHKPSNTKVDKKVEPKSCDKTHTSPPSPAPPVAGPSVFLFPPKPKDTLMISRTPEVTCVVVGVSHEDPEVKFNWYVDGVEVHNAKTKPREEQYNSTYRVVSVLTVLHQDWLNGKEYKCKVSNKQLPSPIEKTISKAKGQPSGQVQLQQSGAELARPGASVKMSCKASGYTFTRYTMHWVKQRPGQGLEWIGYINPSRGYTNYNQKFKDKATLTTDKSSSTAYMQLSSLTSEDSAVYYCARYYDDHYCLDYWGQGTTLTVSSGGGGSGGGGSGGGGSDIVLTQSPAIMSASPGEKVTMTCSASSSVSYMNWYQQKSGTSPKRWIYDTSKLASGVPAHFRGSGSGTSYSLTISGMEAEDAATYYCQQWSSNPFTFGSGTKLEIN

SEQ ID NO: 13 - protein, 235 aa, Artificial Sequence
  light chain of humanized 10B3 antibody
METDTLLLWVLLLWVPGSTGEIVLTQSPATLSLSPGERATLSCSASSSISSNYLHWYQQKPGQAPRLLIYRTSNLASGIPARFSGSGSGTDYTLTISRLEPEDFAVYYCQQGSYIPFTFGQGTKLEIKRTVAAPSVFIFPPSDEQLKSGTASVVCLLNNFYPREAKVQWKVDNALQSGNSQESVTEQDSKDSTYSLSSTLTLSKADYEKHKVYACEVTHQGLSSPVTKSFNRGEC

SEQ ID NO: 14 - protein, 10 aa, Artificial Sequence
  mutated CDR-H1 of 10B3 antibody
GFSFTDFYMY

SEQ ID NO: 15 - protein, 115 aa, Artificial Sequence
  variable heavy chain domain of J519 antibody
EVQLQQSGPELVKPGTSVRISCKTSGYTFTEYTIHWVKQSHGKSLEWIGNINPNNGGTTYNQKFEDKATLTVDKSSSTAYMELRSLTSEDSAVYYCAAGWNFDYWGQGTTLTVSS

SEQ ID NO: 16 - protein, 108 aa, Artificial Sequence
  variable light chain domain Jof J519 antibody
DIVMTQSHKFMSTSVGDRVSIICKASQDVGTAVDWYQQKPGQSPKLLIYWASTRHTGVPDRFTGSGSGTDFTLAITNVQSEDLADYFCQQYNSYPLTFGAGTKLEIKR